European Patent Application EP 4 600 262 A1, published August 13, 2025. Title: Keratin YK93-5, preparation method, and pharmaceutical composition thereof and use thereof. Applicant: Institute of Materia Medica Chinese Academy Of Medical Sciences. The sequence listing filed with the application follows.

SEQUENCE LISTING (2 sequences)

SEQ ID NO: 1 - protein, 507 aa, Manis pentadactyla
MSCRSYRISSGCGVARTFSSCSAVAPKTGSRCCITAAPYRGVSCYRGITGFGSRSLSNLGSCGPRLAVGSFRIGPCGRSFGYRAGGVCGPNPPCITSVSVNESLLAPLNLEIDPNAQCVKQEEKEQIKCLNNRFAAFIDKVRFLEQQNKLLETKWQFYQNRQCCESNLEPLFNGYIETLRREAECAEADSGRLASELNHVQEVLEGFKKKYEEEVALRATAENEFVVLKKDVDCAYLRKSDLEANVEALLEEINFLRRLYDEEIRILHSHISDTSVIVKMDNSRDLNMDCIVAEIKAQYDDIASRSRAEAESWYRTKCEEMKATVIRHGETLRRTKEEINELNRVIQRLTAEIENAKCQRAKLEAAVAEAEQQGEAALNDARCKLAELEAALQKAKQDMACLLKEYQEVMNSKLGLDIEIATYRRLLEGEEHRLCEGVGSVNVCVSSSRGGVSSGGLAFSATSGRQIVSGPVATGGNITLMAPDSCAPCQPRISSFSCGSSRSVRFA

SEQ ID NO: 2 - DNA, 1521 bp, Manis pentadactyla
  source 1..1521: mol_type = genomic DNA
atgagctgtcgtagctatcgcattagtagcggctgcggtgtggcccgcacctttagtagttgcagcgcagtggccccgaaaaccggcagtcgttgctgtattaccgcagccccgtatcgtggcgttagctgctatcgtggcattaccggttttggcagccgtagcctgagtaatctgggtagctgtggcccgcgtctggcagttggtagttttcgcattggtccgtgcggccgtagctttggttatcgcgccggtggcgtgtgtggcccgaatcctccgtgtattaccagcgttagcgtgaatgaaagcctgctggcaccgctgaatctggaaattgatccgaatgcacagtgcgtgaaacaggaagaaaaagaacagattaagtgcctgaataatcgttttgcagcctttattgataaggttcgttttctggaacagcagaataagctgctggaaaccaaatggcagttttatcagaatcgtcagtgctgcgaaagcaatctggaaccgctgtttaatggctatattgaaaccctgcgtcgcgaagcagaatgtgcagaagcagatagcggccgtctggcaagtgaactgaatcatgtgcaggaagtgctggaaggctttaaaaagaaatatgaagaagaggttgccctgcgtgccaccgcagaaaatgaatttgtggtgctgaaaaaagatgtggattgtgcatatctgcgtaaaagtgatctggaagccaatgttgaagcactgctggaagaaattaattttctgcgccgtctgtatgatgaagaaattcgcattctgcatagtcatattagtgataccagtgttattgttaagatggataatagccgtgatctgaatatggattgcattgttgcagaaattaaggcccagtatgatgatattgcaagtcgtagtcgtgccgaagccgaaagctggtatcgcaccaaatgtgaagaaatgaaagcaaccgtgattcgccacggtgaaaccctgcgccgtaccaaagaagaaattaacgaactgaatcgtgttattcagcgtctgaccgcagaaattgaaaatgcaaaatgccagcgcgcaaaactggaagccgccgttgcagaagccgaacagcagggtgaagcagcactgaatgatgcccgttgtaaactggccgaactggaagccgcgctgcagaaagccaaacaggatatggcatgcctgctgaaagaatatcaggaagttatgaatagcaagctgggtctggatattgaaattgccacctatcgccgcctgctggaaggcgaagaacatcgtctgtgcgaaggcgttggcagtgtgaatgtgtgcgttagcagtagtcgtggtggcgtgagcagcggcggtctggcttttagcgccaccagcggccgccagattgttagcggtccggttgccaccggcggtaatattaccctgatggccccggatagctgcgccccgtgtcagcctcgcattagttcattttcttgcggcagcagtcgtagtgttcgctttgcc